European Patent Application EP 4 644 420 A1, published November 5, 2025. Title: ANTIBODY OR ANTIBODY FRAGMENT TARGETING B7-H3, AND USE THEREOF IN FIELD OF CHIMERIC ANTIGEN RECEPTOR IMMUNE CELL THERAPY. Applicant: UNICET BIOTECH CO. LLC. The sequence listing filed with the application follows.

SEQUENCE LISTING (28 sequences)

SEQ ID NO: 1 - protein, 116 aa, unidentified
EVQLQQSGAELVKPGASVKLSCKASGYTFTNYWINWIRQRPGQGLEWIGRIAPGTISTYYNEKFKGRATITEDTSTNTAYLQLSSLTSEDTAVYFCARQDNYFINWGQGTLVTVSS

SEQ ID NO: 2 - protein, 124 aa, unidentified
EFEVQLVESGGGLVKPGGSLKLSCAASGFAFSRYDMSWVRQSPEKRLEWVATISDDGRHTYDRDSVKGRFTISRDNAKNTLYLQMSSLRSEDTALYYCVRHRAITTARFDYWGQGTTVTVSSSR

SEQ ID NO: 3 - protein, 108 aa, unidentified
DIVLTQSPASLSASLGEKVTITCSASSSISSSDLHWYQQKSGTSPRPWIYGTSNLASGVPPRFSGSGSGTSFSLTISSVEAEDVGTYYCQQWFSYPFTFGTGTKLEIK

SEQ ID NO: 4 - protein, 113 aa, unidentified
GCADIVMTQSPSSLSVSLGDTVSITCKASQDIYSNIGWLQQLPGQSFKGLIYHGTNLEDGVPSRFSGSGSGTDYSLTISGLESEDFADYYCLQYVQFPYTFGGGTKLEIKASG

SEQ ID NO: 5 - DNA, 348 bp, unidentified
  source 1..348: mol_type = other DNA
gaagtgcagctccagcagagcggagcagaactggtgaagccaggagccagcgtgaagctgtcttgcaaggccagcggctacaccttcaccaactactggatcaattggatcagacagaggccaggacagggactcgagtggattggcagaatcgccccaggcaccatcagcacctactacaacgagaagttcaagggcagggccaccatcaccgaggataccagcaccaacaccgcctacctccagctgtctagcctgacaagcgaggacacagccgtgtacttttgcgccaggcaggacaactacttcatcaattggggccagggaaccctggtgacagtgtccagc

SEQ ID NO: 6 - DNA, 372 bp, unidentified
  source 1..372: mol_type = other DNA
gagttcgaggtgcagctggtggagagcggaggtgggctagttaaacccggcggctccttgaagctgtcatgcgctgcttctgggtttgcgttctcccgctacgacatgagttgggtgcgccagagccctgaaaagcgcctggagtgggtcgccaccattagcgatgacggcagacacacctacgacagggatagcgtaaagggtcgcttcaccatctctcgtgacaacgccaagaacacgctttacctgcagatgtcctctctgcgctcggaggacaccgcgctctactactgcgtgcgacatcgcgccatcactactgcacggttcgactattggggccagggcaccacagtcaccgtgtcgtcctcccgt

SEQ ID NO: 7 - DNA, 324 bp, unidentified
  source 1..324: mol_type = other DNA
gacattgttcttacacaatctccggccagcctctctgcgagcctcggggaaaaggtgacaatcacttgttccgcatcatcaagtatctccagctctgacctgcactggtatcagcagaaaagtggcaccagtccgaggccgtggatctatggcactagcaatcttgcgtcaggagtcccaccccgctttagtggcagtggatcagggacatcattcagtctgacaatctctagcgtcgaggcggaggatgtcggcacatattactgccaacagtggttttcttatcctttcacatttggtacgggcacgaaactggaaataaaa

SEQ ID NO: 8 - DNA, 339 bp, unidentified
  source 1..339: mol_type = other DNA
gggtgcgcggacatcgtgatgacccagagtccgtcgtctctgagcgtctcgctcggcgacaccgtgagcatcacttgtaaagcttcccaggacatctactccaacatcggttggctacaacagctgcccggacagtccttcaagggcctgatttaccacgggaccaacctggaggacggcgttccttcccgcttcagcggctccggctccggtacagattactctctgaccatttctggccttgagagcgaagactttgccgattactactgcctgcagtacgtgcagttcccctataccttcggcggtggcactaagttggagatcaaggcctcaggc

SEQ ID NO: 9 - protein, 5 aa, unidentified
NYWIN

SEQ ID NO: 10 - protein, 17 aa, unidentified
RIAPGTISTYYNEKFKG

SEQ ID NO: 11 - protein, 7 aa, unidentified
QDNYFIN

SEQ ID NO: 12 - protein, 12 aa, unidentified
SASSSISSSDLH

SEQ ID NO: 13 - protein, 7 aa, unidentified
GTSNLAS

SEQ ID NO: 14 - protein, 9 aa, unidentified
QQWFSYPFT

SEQ ID NO: 15 - protein, 5 aa, unidentified
RYDMS

SEQ ID NO: 16 - protein, 17 aa, unidentified
TISDDGRHTYDRDSVKG

SEQ ID NO: 17 - protein, 11 aa, unidentified
HRAITTARFDY

SEQ ID NO: 18 - protein, 11 aa, unidentified
KASQDIYSNIG

SEQ ID NO: 19 - protein, 7 aa, unidentified
HGTNLED

SEQ ID NO: 20 - protein, 9 aa, unidentified
LQYVQFPYT

SEQ ID NO: 21 - DNA, 165 bp, unidentified
  source 1..165: mol_type = other DNA
ttcgtgccggtcttcctgccagcgaagcccaccacgacgccagcgccgcgaccaccaacaccggcgcccaccatcgcgtcgcagcccctgtccctgcgcccagaggcgtgccggccagcggcggggggcgcagtgcacacgagggggctggacttcgcctgtgat

SEQ ID NO: 22 - DNA, 84 bp, unidentified
  source 1..84: mol_type = other DNA
atctacatctgggcgcccttggccgggacttgtggggtccttctcctgtcactggttatcaccctttactgcaaccacaggaac

SEQ ID NO: 23 - DNA, 66 bp, unidentified
  source 1..66: mol_type = other DNA
atggccctgattgtgctggggggcgtcgccggcctcctgcttttcattgggctaggcatcttcttc

SEQ ID NO: 24 - DNA, 141 bp, unidentified
  source 1..141: mol_type = other DNA
cgtttctctgttgttaaacggggcagaaagaagctcctgtatatattcaaacaaccatttatgagaccagtacaaactactcaagaggaagatggctgtagctgccgatttccagaagaagaagaaggaggatgtgaactg

SEQ ID NO: 25 - DNA, 123 bp, unidentified
  source 1..123: mol_type = other DNA
aggagtaagaggagcaggctcctgcacagtgactacatgaacatgactccccgccgccccgggcccacccgcaagcattaccagccctatgccccaccacgcgacttcgcagcctatcgctcc

SEQ ID NO: 26 - DNA, 336 bp, unidentified
  source 1..336: mol_type = other DNA
agagtgaagttcagcaggagcgcagacgcccccgcgtaccagcagggccagaaccagctctataacgagctcaatctaggacgaagagaggagtacgatgttttggacaagagacgtggccgggaccctgagatggggggaaagccgagaaggaagaaccctcaggaaggcctgtacaatgaactgcagaaagataagatggcggaggcctacagtgagattgggatgaaaggcgagcgccggaggggcaaggggcacgatggcctttaccagggtctcagtacagccaccaaggacacctacgacgcccttcacatgcaggccctgccccctcgc

SEQ ID NO: 27 - DNA, 1638 bp, synthetic construct
  source 1..1638: mol_type = other DNA
atggagacagacacactcctgctatgggtgctgctgctctgggttccaggttccacaggtgacgaggtgcagctgcaacagagcggtgccgagctggtgaagcccggcgcgtccgttaagctatcatgcaaagcgtccggctacacgttcaccaactattggattaattggatccggcagaggcccggacagggcctcgaatggatcggtcgcatcgcgcccgggacgatttccacttattacaacgagaaatttaagggccgcgccaccataactgaggatacctcgaccaacaccgcctacctgcagctttcgtccctgacctcggaggacacggccgtgtacttctgtgctcgccaggacaactactttattaactggggccagggtactcttgtcaccgtcagctcggggggcggcggctccggaggcggtggttcaggcgggggaggctccgacatcgtgctgacccagagccctgcttccttgagcgcatctctgggcgagaaggtaactatcacctgctctgcttcgtcctctatctcttctagtgacctgcactggtaccagcagaagtccggtacaagtcctcgtccgtggatctacggcaccagcaacctggcctctggcgtcccaccgcgcttctctggaagcgggtccgggacttccttttcgctcacaatcagctccgtggaggctgaagatgtgggcacctactactgtcagcagtggttcagctaccccttcaccttcggcaccggcaccaagctggagatcaaggcggccgcattcgtgccggtcttcctgccagcgaagcccaccacgacgccagcgccgcgaccaccaacaccggcgcccaccatcgcgtcgcagcccctgtccctgcgcccagaggcgtgccggccagcggcggggggcgcagtgcacacgagggggctggacttcgcctgtgatatctacatctgggcgcccttggccgggacttgtggggtccttctcctgtcactggttatcaccctttactgcaaccacaggaacaggagtaagaggagcaggctcctgcacagtgactacatgaacatgactccccgccgccccgggcccacccgcaagcattaccagccctatgccccaccacgcgacttcgcagcctatcgctcccgtttctctgttgttaaacggggcagaaagaagctcctgtatatattcaaacaaccatttatgagaccagtacaaactactcaagaggaagatggctgtagctgccgatttccagaagaagaagaaggaggatgtgaactgagagtgaagttcagcaggagcgcagacgcccccgcgtaccagcagggccagaaccagctctataacgagctcaatctaggacgaagagaggagtacgatgttttggacaagagacgtggccgggaccctgagatggggggaaagccgagaaggaagaaccctcaggaaggcctgtacaatgaactgcagaaagataagatggcggaggcctacagtgagattgggatgaaaggcgagcgccggaggggcaaggggcacgatggcctttaccagggtctcagtacagccaccaaggacacctacgacgcccttcacatgcaggccctgccccctcgc

SEQ ID NO: 28 - DNA, 1677 bp, synthetic construct
  source 1..1677: mol_type = other DNA
atggagacagacacactcctgctatgggtgctgctgctctgggttccaggttccacaggtgacgagttcgaggtgcagctggtggagagcggaggtgggctagttaaacccggcggctccttgaagctgtcatgcgctgcttctgggtttgcgttctcccgctacgacatgagttgggtgcgccagagccctgaaaagcgcctggagtgggtcgccaccattagcgatgacggcagacacacctacgacagggatagcgtaaagggtcgcttcaccatctctcgtgacaacgccaagaacacgctttacctgcagatgtcctctctgcgctcggaggacaccgcgctctactactgcgtgcgacatcgcgccatcactactgcacggttcgactattggggccagggcaccacagtcaccgtgtcgtcctcccgtgggggcggcggctccggaggcggtggttcaggcgggggaggctccgggtgcgcggacatcgtgatgacccagagtccgtcgtctctgagcgtctcgctcggcgacaccgtgagcatcacttgtaaagcttcccaggacatctactccaacatcggttggctacaacagctgcccggacagtccttcaagggcctgatttaccacgggaccaacctggaggacggcgttccttcccgcttcagcggctccggctccggtacagattactctctgaccatttctggccttgagagcgaagactttgccgattactactgcctgcagtacgtgcagttcccctataccttcggcggtggcactaagttggagatcaaggcctcaggcgcggccgcattcgtgccggtcttcctgccagcgaagcccaccacgacgccagcgccgcgaccaccaacaccggcgcccaccatcgcgtcgcagcccctgtccctgcgcccagaggcgtgccggccagcggcggggggcgcagtgcacacgagggggctggacttcgcctgtgatatctacatctgggcgcccttggccgggacttgtggggtccttctcctgtcactggttatcaccctttactgcaaccacaggaacaggagtaagaggagcaggctcctgcacagtgactacatgaacatgactccccgccgccccgggcccacccgcaagcattaccagccctatgccccaccacgcgacttcgcagcctatcgctcccgtttctctgttgttaaacggggcagaaagaagctcctgtatatattcaaacaaccatttatgagaccagtacaaactactcaagaggaagatggctgtagctgccgatttccagaagaagaagaaggaggatgtgaactgagagtgaagttcagcaggagcgcagacgcccccgcgtaccagcagggccagaaccagctctataacgagctcaatctaggacgaagagaggagtacgatgttttggacaagagacgtggccgggaccctgagatggggggaaagccgagaaggaagaaccctcaggaaggcctgtacaatgaactgcagaaagataagatggcggaggcctacagtgagattgggatgaaaggcgagcgccggaggggcaaggggcacgatggcctttaccagggtctcagtacagccaccaaggacacctacgacgcccttcacatgcaggccctgccccctcgc